European Patent Specification EP 3 541 829 B1, published July 16, 2025. Title: Substances for targeting various selected organs or tissues. Applicant: Academisch Ziekenhuis Leiden BioMarin Technologies B.V. Application 17804132.3. The sequence listing filed with the application follows.

SEQUENCE LISTING (83 sequences)

SEQ ID NO: 1 - protein, 7 aa, Artificial Sequence
  Randomly generated peptide
LTLPWSK

SEQ ID NO: 2 - protein, 7 aa, Artificial Sequence
  Randomly generated peptide
VKHKSLD

SEQ ID NO: 3 - protein, 7 aa, Artificial Sequence
  Randomly generated peptide
KYMSSHA

SEQ ID NO: 4 - protein, 7 aa, Artificial Sequence
  Randomly generated peptide
VSPSKSF

SEQ ID NO: 5 - protein, 7 aa, Artificial Sequence
  Randomly generated peptide
YETKSES

SEQ ID NO: 6 - protein, 7 aa, Artificial Sequence
  Randomly generated peptide
DPRTQPH

SEQ ID NO: 7 - protein, 7 aa, Artificial Sequence
  Randomly generated peptide
KDPRPAL

SEQ ID NO: 8 - protein, 7 aa, Artificial Sequence
  Randomly generated peptide
LKSAGNN

SEQ ID NO: 9 - protein, 7 aa, Artificial Sequence
  Randomly generated peptide
IAWNKQG

SEQ ID NO: 10 - protein, 7 aa, Artificial Sequence
  Randomly generated peptide
YGTGNNY

SEQ ID NO: 11 - protein, 7 aa, Artificial Sequence
  Randomly generated peptide
SRFQLPQ

SEQ ID NO: 12 - protein, 7 aa, Artificial Sequence
  Randomly generated peptide
LPDAYHV

SEQ ID NO: 13 - protein, 7 aa, Artificial Sequence
  Randomly generated peptide
KTGHAHL

SEQ ID NO: 14 - protein, 7 aa, Artificial Sequence
  Randomly generated peptide
QVRSNTT

SEQ ID NO: 15 - protein, 7 aa, Artificial Sequence
  Randomly generated peptide
SLFKNSR

SEQ ID NO: 16 - protein, 7 aa, Artificial Sequence
  Randomly generated peptide
RADFYTT

SEQ ID NO: 17 - protein, 7 aa, Artificial Sequence
  Randomly generated peptide
RENTNHT

SEQ ID NO: 18 - protein, 7 aa, Artificial Sequence
  Randomly generated peptide
WNEDHTW

SEQ ID NO: 19 - protein, 7 aa, Artificial Sequence
  Randomly generated peptide
LLGHTNN

SEQ ID NO: 20 - protein, 7 aa, Artificial Sequence
  Randomly generated peptide
FSHTYRV

SEQ ID NO: 21 - protein, 7 aa, Artificial Sequence
  Randomly generated peptide
TYSPTEV

SEQ ID NO: 22 - protein, 7 aa, Artificial Sequence
  Randomly generated peptide
TLQDQAT

SEQ ID NO: 23 - protein, 7 aa, Artificial Sequence
  Randomly generated peptide
MQHSMRV

SEQ ID NO: 24 - protein, 7 aa, Artificial Sequence
  Randomly generated peptide
LNSLFGS

SEQ ID NO: 25 - protein, 7 aa, Artificial Sequence
  Randomly generated peptide
QLFPLFR

SEQ ID NO: 26 - protein, 7 aa, Artificial Sequence
  Randomly generated peptide
SNNFVEH

SEQ ID NO: 27 - protein, 7 aa, Artificial Sequence
  Randomly generated peptide
LPDAYHV

SEQ ID NO: 28 - protein, 7 aa, Artificial Sequence
  Randomly generated peptide
MTNPNSW

SEQ ID NO: 29 - protein, 7 aa, Artificial Sequence
  Randomly generated peptide
LSVGSEA

SEQ ID NO: 30 - protein, 7 aa, Artificial Sequence
  Randomly generated peptide
VSTTIMS

SEQ ID NO: 31 - protein, 7 aa, Artificial Sequence
  Randomly generated peptide
NNSLMYW

SEQ ID NO: 32 - protein, 7 aa, Artificial Sequence
  Randomly generated peptide
NAPGPQN

SEQ ID NO: 33 - protein, 7 aa, Artificial Sequence
  Randomly generated peptide
GMNFTSF

SEQ ID NO: 34 - protein, 7 aa, Artificial Sequence
  Randomly generated peptide
SPLTTGY

SEQ ID NO: 35 - protein, 7 aa, Artificial Sequence
  Randomly generated peptide
SIYSMYP

SEQ ID NO: 36 - protein, 7 aa, Artificial Sequence
  Randomly generated peptide
NSSRLPV

SEQ ID NO: 37 - protein, 7 aa, Artificial Sequence
  Randomly generated peptide
VRNNTWS

SEQ ID NO: 38 - protein, 7 aa, Artificial Sequence
  Randomly generated peptide
QHTVGSL

SEQ ID NO: 39 - protein, 7 aa, Artificial Sequence
  Randomly generated peptide
MHPQWQY

SEQ ID NO: 40 - protein, 7 aa, Artificial Sequence
  Randomly generated peptide
TPGSTQE

SEQ ID NO: 41 - protein, 7 aa, Artificial Sequence
  Randomly generated peptide
SLNTTVT

SEQ ID NO: 42 - protein, 7 aa, Artificial Sequence
  Randomly generated peptide
QTTMWNW

SEQ ID NO: 43 - protein, 7 aa, Artificial Sequence
  Randomly generated peptide
QTTLCCL

SEQ ID NO: 44 - protein, 7 aa, Artificial Sequence
  Randomly generated peptide
MISPSHT

SEQ ID NO: 45 - protein, 7 aa, Artificial Sequence
  Randomly generated peptide
MSASNLN

SEQ ID NO: 46 - protein, 7 aa, Artificial Sequence
  Randomly generated peptide
GSLFVSM

SEQ ID NO: 47 - protein, 7 aa, Artificial Sequence
  Randomly generated peptide
LNSLFGS

SEQ ID NO: 48 - protein, 7 aa, Artificial Sequence
  Randomly generated peptide
VGSTVSH

SEQ ID NO: 49 - protein, 7 aa, Artificial Sequence
  Randomly generated peptide
LLPLTSV

SEQ ID NO: 50 - protein, 7 aa, Artificial Sequence
  Randomly generated peptide
QMDARKY

SEQ ID NO: 51 - protein, 7 aa, Artificial Sequence
  Randomly generated peptide
HLNSEKT

SEQ ID NO: 52 - protein, 7 aa, Artificial Sequence
  Randomly generated peptide
INTESKQ

SEQ ID NO: 53 - protein, 7 aa, Artificial Sequence
  Randomly generated peptide
VTQNKDM

SEQ ID NO: 54 - protein, 7 aa, Artificial Sequence
  Randomly generated peptide
RNNAPWI

SEQ ID NO: 55 - protein, 7 aa, Artificial Sequence
  Randomly generated peptide
LNRQPNM

SEQ ID NO: 56 - protein, 7 aa, Artificial Sequence
  Randomly generated peptide
IVPSLQR

SEQ ID NO: 57 - protein, 7 aa, Artificial Sequence
  Randomly generated peptide
NNSLMYW

SEQ ID NO: 58 - protein, 7 aa, Artificial Sequence
  Randomly generated peptide
SLLSVHR

SEQ ID NO: 59 - protein, 7 aa, Artificial Sequence
  Randomly generated peptide
WHTGSKI

SEQ ID NO: 60 - protein, 7 aa, Artificial Sequence
  Randomly generated peptide
SIYSMYP

SEQ ID NO: 61 - protein, 7 aa, Artificial Sequence
  Randomly generated peptide
QHTVGSL

SEQ ID NO: 62 - protein, 7 aa, Artificial Sequence
  Randomly generated peptide
DRSLNHH

SEQ ID NO: 63 - protein, 7 aa, Artificial Sequence
  Randomly generated peptide
MNRANLK

SEQ ID NO: 64 - DNA, 57 bp, Artificial Sequence
  Primer for phage
aatgatacggcgaccaccgagatctacacttcctttagtggtacctttctattctca

SEQ ID NO: 65 - DNA, 60 bp, Artificial Sequence
  Primer for phage with variable barcode region
  misc_feature (28)..(36): n is a, c, g, or t
caagcagaagacggcatacgagatcggnnnnnnnnnatgggattttgctaaacaactttc

SEQ ID NO: 66 - DNA, 36 bp, Artificial Sequence
  Primer for sequencing
acacttcctttagtggtacctttctattctcactct

SEQ ID NO: 67 - RNA, 23 nt, Artificial Sequence
  Antisense oligonucleotide for human DMD exon 45
ugccgcugcccaaugggauccug

SEQ ID NO: 68 - RNA, 20 nt, Artificial Sequence
  Antisense oligonucleotide for murine DMD exon 23
ggccaaaccucggcuuaccu

SEQ ID NO: 69 - protein, 4 aa, Artificial Sequence
  Nuclear localisation signal
KKKR

SEQ ID NO: 70 - protein, 4 aa, Artificial Sequence
  Nuclear localisation signal
KKRK

SEQ ID NO: 71 - protein, 5 aa, Artificial Sequence
  Nuclear localisation signal
KKKRK

SEQ ID NO: 72 - protein, 4 aa, Artificial Sequence
  Nuclear localisation signal
KKRS

SEQ ID NO: 73 - protein, 4 aa, Artificial Sequence
  Nuclear localisation signal
KRSK

SEQ ID NO: 74 - protein, 5 aa, Artificial Sequence
  Nuclear localisation signal
KKRSK

SEQ ID NO: 75 - protein, 4 aa, Artificial Sequence
  Nuclear localisation signal
KSRK

SEQ ID NO: 76 - protein, 4 aa, Artificial Sequence
  Nuclear localisation signal
SRKR

SEQ ID NO: 77 - protein, 4 aa, Artificial Sequence
  Nuclear localisation signal
RKRK

SEQ ID NO: 78 - protein, 5 aa, Artificial Sequence
  Nuclear localisation signal
KSRKR

SEQ ID NO: 79 - protein, 5 aa, Artificial Sequence
  Nuclear localisation signal
SRKRK

SEQ ID NO: 80 - protein, 6 aa, Artificial Sequence
  Nuclear localisation signal
KSRKRK

SEQ ID NO: 81 - protein, 7 aa, Artificial Sequence
  Nuclear localisation signal
PKKKRKV

SEQ ID NO: 82 - protein, 7 aa, Artificial Sequence
  Nuclear localisation signal
GKKRSKV

SEQ ID NO: 83 - protein, 7 aa, Artificial Sequence
  Nuclear localisation signal
KSRKRKL